European Patent Application EP 4 620 973 A1, published September 24, 2025. Title: ANTIBODIES TARGETING CELL SURFACE DEPOSITED COMPLEMENT PROTEIN C3d AND USE THEREOF. Applicant: THE UNITED STATES OF AMERICA, AS REPRESENTED BY THE SECRETARY, DEPARTMENT OF HEALTH AND HUMAN SERVICES. Application US. The sequence listing filed with the application follows.

SEQUENCE LISTING (41 sequences)

SEQ ID NO: 1 - protein, 112 aa, Synthetic construct
QSVEESRGRLVTPGTPLTLTCTVSGIDLSSSAITWVRQAPGKGLEWIGMISTDGATYYANWAKGRFTFSKTSTTADLKITSPTTEDTATYFCARGLTNFSIWGPGTLVTVSS

SEQ ID NO: 2 - protein, 112 aa, Synthetic construct
QPVLTQSPSASAALGASAKLTCTLSSAHKTYTIAWYQQQPGESPRYLMLLKSDGSYTRGPGVPDRFSGSSSGADRYLIIPSVQADDEAGYYCGADYNGGYVFGGGTQLTVTG

SEQ ID NO: 3 - protein, 121 aa, Synthetic construct
QSVEESGGRLVTPGTPLTLTCTVSGFSLSSYAMTWVRQAPGKGLEWIGVIGTSGMRYYANWAKGRFTISKTSTTVDLKITSPTTEDTATYFCARANFYVGNDESTDAFDPWGPGTLVTVSS

SEQ ID NO: 4 - protein, 110 aa, Synthetic construct
ALVMTQTPPSLSASVGETVRIRCLASEDIYNTISWYQQKPGKPPTLLIYGASNLKSGVPPRFSGSGSGTDYTLTIGGVQSEDAATYYCLGGYSYSSTGLTFGAGTKVEIK

SEQ ID NO: 5 - protein, 120 aa, Synthetic construct
QKQLVESGGRLVTPGGSLTLTCTISGIDLNTYGMTWVRQAPGKGLEYIGIIVSSGNTYYANWAQGRFTISKTSTTVDLKMTSLTASDTATYFCARGLGRAYSSGYGMDGWGPGTLVTVSS

SEQ ID NO: 6 - protein, 108 aa, Synthetic construct
DPVLTQTPSSTSAAVGGTVTIKCQASQNIYTSLAWYQQKPGQPPKLLIYGASNLASGVPSRFKGSRSGTEYTLTISGVEREDAATYYCLGSYTQIDTTFGGGTKLEIK

SEQ ID NO: 7 - protein, 120 aa, Synthetic construct
QSLEESGGRLVTPGTPLTLTCTVSGFSLSRYTMAWVRQAPGKGLEYIGWIDSSGSTYYASWAKGRFTISKTSSTTVDLKMTSLTTEDTATYFCASGNDGGDPLYYGMDPWGPGTLVTVSS

SEQ ID NO: 8 - protein, 108 aa, Synthetic construct
DGVMTQTPSSTSAAVGGTVTIKCQASQSIRSWLSWYQQKPGQPPKLLIYEASKLASGVPSRFKGSRSGTEYTLAISGVQREDAATYYCLGSIASDDTAFGAGTNVEIK

SEQ ID NO: 9 - protein, 120 aa, Synthetic construct
QSLEESGGRLVTPGTPLTLTCTVSGFSLSTYTLGWVRQAPGKGLEYIGWIDSSGSAYYASWAKGRFTISKASSTTVDLKMAGLTTEDTATYFCASGNTGGDPLYYGMDPWGPGTLVTVSS

SEQ ID NO: 10 - protein, 108 aa, Synthetic construct
DPVLTQTPSSTSAAVGGTVTIKCQASQNIGRWLAWYQQKPGQPPKLLIYRASDLASGVPSRFKGSGSGTQFTLTISGVQREDAATYYCLGSYSSSDSAFGGGTEVVVK

SEQ ID NO: 11 - protein, 5 aa, Synthetic construct
SSAIT

SEQ ID NO: 12 - protein, 16 aa, Synthetic construct
MISTDGATYYANWAKG

SEQ ID NO: 13 - protein, 7 aa, Synthetic construct
GLTNFSI

SEQ ID NO: 14 - protein, 12 aa, Synthetic construct
TLSSAHKTYTIA

SEQ ID NO: 15 - protein, 9 aa, Synthetic construct
LKSDGSYTR

SEQ ID NO: 16 - protein, 9 aa, Synthetic construct
GADYNGGYV

SEQ ID NO: 17 - protein, 5 aa, Synthetic construct
SYAMT

SEQ ID NO: 18 - protein, 16 aa, Synthetic construct
VIGTSGMRYYANWAKG

SEQ ID NO: 19 - protein, 16 aa, Synthetic construct
ANFYVGNDESTDAFDP

SEQ ID NO: 20 - protein, 11 aa, Synthetic construct
LASEDIYNTIS

SEQ ID NO: 21 - protein, 7 aa, Synthetic construct
GASNLKS

SEQ ID NO: 22 - protein, 12 aa, Synthetic construct
LGGYSYSSTGLT

SEQ ID NO: 23 - protein, 5 aa, Synthetic construct
TYGMT

SEQ ID NO: 24 - protein, 16 aa, Synthetic construct
IIVSSGNTYYANWAQG

SEQ ID NO: 25 - protein, 14 aa, Synthetic construct
GLGRAYSSGYGMDG

SEQ ID NO: 26 - protein, 11 aa, Synthetic construct
QASQNIYTSLA

SEQ ID NO: 27 - protein, 7 aa, Synthetic construct
GASNLAS

SEQ ID NO: 28 - protein, 10 aa, Synthetic construct
LGSYTQIDTT

SEQ ID NO: 29 - protein, 5 aa, Synthetic construct
RYTMA

SEQ ID NO: 30 - protein, 16 aa, Synthetic construct
WIDSSGSTYYASWAKG

SEQ ID NO: 31 - protein, 14 aa, Synthetic construct
GNDGGDPLYYGMDP

SEQ ID NO: 32 - protein, 11 aa, Synthetic construct
QASQSIRSWLS

SEQ ID NO: 33 - protein, 7 aa, Synthetic construct
EASKLAS

SEQ ID NO: 34 - protein, 10 aa, Synthetic construct
LGSIASDDTA

SEQ ID NO: 35 - protein, 5 aa, Synthetic construct
TYTLG

SEQ ID NO: 36 - protein, 16 aa, Synthetic construct
WIDSSGSAYYASWAKG

SEQ ID NO: 37 - protein, 14 aa, Synthetic construct
GNTGGDPLYYGMDP

SEQ ID NO: 38 - protein, 11 aa, Synthetic construct
QASQNIGRWLA

SEQ ID NO: 39 - protein, 7 aa, Synthetic construct
RASDLAS

SEQ ID NO: 40 - protein, 10 aa, Synthetic construct
LGSYSSSDSA

SEQ ID NO: 41 - DNA, 24 bp, Synthetic construct
  source 1..24: mol_type = other DNA
gaagactgayggagccttaggttg